European Patent Application EP 4 364 746 A1, published May 8, 2024. Title: UNIVERSAL CAR-T CELL TARGETING IL13Rα2, PREPARATION METHOD THEREFOR AND APPLICATION THEREOF. Applicant: NINGBO T-MAXIMUM BIOPHARMACEUTICALS CO., LTD. The sequence listing filed with the application follows.

SEQUENCE LISTING (245 sequences)

SEQ ID NO: 1 - protein, 6 aa, Artificial Sequence
  Mu01 HCDR1; Hu01 HCDR1;
SRNGMS

SEQ ID NO: 2 - protein, 17 aa, Artificial Sequence
  Mu01 HCDR2; Hu01 HCDR2;
TVSSGGSYIYYADSVKG

SEQ ID NO: 3 - protein, 13 aa, Artificial Sequence
  Mu01 HCDR3; Hu01 HCDR3;
QGTTALATRFFDV

SEQ ID NO: 4 - protein, 29 aa, Artificial Sequence
  Mu01 HFR1; Hu01 HFR1
  misc_feature (10)..(10): Xaa = Asp or Gly
  misc_feature (13)..(13): Xaa = Gln or Arg
  misc_feature (19)..(19): Xaa = Gln or Arg
EVQLVESGGXLVXPGGSLXLSCAASGFTF

SEQ ID NO: 5 - protein, 14 aa, Artificial Sequence
  Mu01 HFR2; Hu01 HFR2
  misc_feature (5)..(5): Xaa = Ala or Thr
  misc_feature (7)..(7): Xaa = Asp or Gly
  misc_feature (8)..(8): Xaa = Lys or Arg
  misc_feature (9)..(9): Xaa = Gly or Arg
WVRQXPXXXLEWVA

SEQ ID NO: 6 - protein, 32 aa, Artificial Sequence
  Mu01 HFR3; Hu01 HFR3
  misc_feature (10)..(10): Xaa = Lys or Arg
  misc_feature (12)..(12): Xaa = Ser or Thr
  misc_feature (18)..(18): Xaa = Asn or Ser
  misc_feature (21)..(21): Xaa = Lys or Arg
  misc_feature (22)..(22): Xaa = Ala or Ser
  misc_feature (27)..(27): Xaa = Met or Val
RFTISRDNAXNXLYLQMXSLXXEDTAXYYCAR

SEQ ID NO: 7 - protein, 11 aa, Artificial Sequence
  Mu01 HFR4; Hu01 HFR4
  misc_feature (3)..(3): Xaa = Ala or Gln
  misc_feature (6)..(6): Xaa = Leu or Thr
WGXGTXVTVSS

SEQ ID NO: 8 - protein, 29 aa, Artificial Sequence
  Mu01 HFR1
EVQLVESGGDLVRPGGSLQLSCAASGFTF

SEQ ID NO: 9 - protein, 14 aa, Artificial Sequence
  Mu01 HFR2
WVRQTPDRRLEWVA

SEQ ID NO: 10 - protein, 32 aa, Artificial Sequence
  Mu01 HFR3
RFTISRDNARNTLYLQMSSLKSEDTAMYYCAR

SEQ ID NO: 11 - protein, 11 aa, Artificial Sequence
  Mu01 HFR4
WGAGTTVTVSS

SEQ ID NO: 12 - protein, 29 aa, Artificial Sequence
  Hu01 HFR1
EVQLVESGGGLVQPGGSLRLSCAASGFTF

SEQ ID NO: 13 - protein, 14 aa, Artificial Sequence
  Hu01 HFR2
WVRQAPGKGLEWVA

SEQ ID NO: 14 - protein, 32 aa, Artificial Sequence
  Hu01 HFR3
RFTISRDNAKNSLYLQMNSLRAEDTAVYYCAR

SEQ ID NO: 15 - protein, 11 aa, Artificial Sequence
  Hu01 HFR4
WGQGTLVTVSS

SEQ ID NO: 16 - protein, 122 aa, Artificial Sequence
  Mu01 VH
EVQLVESGGDLVRPGGSLQLSCAASGFTFSRNGMSWVRQTPDRRLEWVATVSSGGSYIYYADSVKGRFTISRDNARNTLYLQMSSLKSEDTAMYYCARQGTTALATRFFDVWGAGTTVTVSS

SEQ ID NO: 17 - protein, 122 aa, Artificial Sequence
  Hu01 VH
EVQLVESGGGLVQPGGSLRLSCAASGFTFSRNGMSWVRQAPGKGLEWVATVSSGGSYIYYADSVKGRFTISRDNAKNSLYLQMNSLRAEDTAVYYCARQGTTALATRFFDVWGQGTLVTVSS

SEQ ID NO: 18 - protein, 122 aa, Artificial Sequence
  Mu01 VH; Hu01 VH
  misc_feature (10)..(10): Xaa = Asp or Gly
  misc_feature (13)..(13): Xaa = Gln or Arg
  misc_feature (19)..(19): Xaa = Gln or Arg
  misc_feature (40)..(40): Xaa = Ala or Thr
  misc_feature (42)..(42): Xaa = Asp or Gly
  misc_feature (43)..(43): Xaa = Lys or Arg
  misc_feature (44)..(44): Xaa = Gly or Arg
  misc_feature (76)..(76): Xaa = Lys or Arg
  misc_feature (78)..(78): Xaa = Ser or Thr
  misc_feature (84)..(84): Xaa = Asn or Ser
  misc_feature (87)..(87): Xaa = Lys or Arg
  misc_feature (88)..(88): Xaa = Ala or Ser
  misc_feature (93)..(93): Xaa = Met or Val
  misc_feature (114)..(114): Xaa = Ala or Gln
  misc_feature (117)..(117): Xaa = Leu or Thr
EVQLVESGGXLVXPGGSLXLSCAASGFTFSRNGMSWVRQXPXXXLEWVATVSSGGSYIYYADSVKGRFTISRDNAXNXLYLQMXSLXXEDTAXYYCARQGTTALATRFFDVWGXGTXVTVSS

SEQ ID NO: 19 - protein, 11 aa, Artificial Sequence
  Mu01 LCDR1; Hu01 LCDR1;
KASQDVGTAVA

SEQ ID NO: 20 - protein, 7 aa, Artificial Sequence
  Mu01 LCDR2; Hu01 LCDR2;
SASYRST

SEQ ID NO: 21 - protein, 9 aa, Artificial Sequence
  Mu01 LCDR3; Hu01 LCDR3;
QHHYSAPWT

SEQ ID NO: 22 - protein, 23 aa, Artificial Sequence
  Mu01 LFR1; Hu01 LFR1
  misc_feature (3)..(3): Xaa = Gln or Val
  misc_feature (8)..(8): Xaa = His or Pro
  misc_feature (9)..(9): Xaa = Lys or Ser
  misc_feature (10)..(10): Xaa = Phe or Ser
  misc_feature (11)..(11): Xaa = Ile or Leu
  misc_feature (13)..(13): Xaa = Ala or Thr
  misc_feature (20)..(20): Xaa = Ser or Thr
DIXMTQSXXXXSXSVGDRVXITC

SEQ ID NO: 23 - protein, 15 aa, Artificial Sequence
  Mu01 LFR2; Hu01 LFR2
  misc_feature (5)..(5): Xaa = Ile or Lys
  misc_feature (8)..(8): Xaa = Lys or Gln
  misc_feature (9)..(9): Xaa = Ala or Ser
WYQQXPGXXPKLLIY

SEQ ID NO: 24 - protein, 32 aa, Artificial Sequence
  Mu01 LFR3; Hu01 LFR3
  misc_feature (2)..(2): Xaa = Ile or Val
  misc_feature (4)..(4): Xaa = Asp or Ser
  misc_feature (7)..(7): Xaa = Ser or Thr
  misc_feature (16)..(16): Xaa = Ser or Thr
  misc_feature (17)..(17): Xaa = Phe or Leu
  misc_feature (18)..(18): Xaa = Ile or Thr
  misc_feature (22)..(22): Xaa = Leu or Val
  misc_feature (24)..(24): Xaa = Ala or Pro
  misc_feature (27)..(27): Xaa = Phe or Leu
  misc_feature (29)..(29): Xaa = Leu or Thr
GXPXRFXGSGSGTDFXXXISSXQXEDXAXYYC

SEQ ID NO: 25 - protein, 10 aa, Artificial Sequence
  Mu01 LFR4; Hu01 LFR4
  misc_feature (6)..(6): Xaa = Lys or Thr
  misc_feature (7)..(7): Xaa = Leu or Val
  misc_feature (8)..(8): Xaa = Asp or Glu
FGGGTXXXIK

SEQ ID NO: 26 - protein, 23 aa, Artificial Sequence
  Mu01 LFR1
DIVMTQSHKFISTSVGDRVSITC

SEQ ID NO: 27 - protein, 15 aa, Artificial Sequence
  Mu01 LFR2
WYQQIPGQSPKLLIY

SEQ ID NO: 28 - protein, 32 aa, Artificial Sequence
  Mu01 LFR3
GIPDRFTGSGSGTDFSFIISSVQAEDLALYYC

SEQ ID NO: 29 - protein, 10 aa, Artificial Sequence
  Mu01 LFR4
FGGGTTLDIK

SEQ ID NO: 30 - protein, 23 aa, Artificial Sequence
  Hu01 LFR1
DIQMTQSPSSLSASVGDRVTITC

SEQ ID NO: 31 - protein, 15 aa, Artificial Sequence
  Hu01 LFR2
WYQQKPGKAPKLLIY

SEQ ID NO: 32 - protein, 32 aa, Artificial Sequence
  Hu01 LFR3
GVPSRFSGSGSGTDFTLTISSLQPEDFATYYC

SEQ ID NO: 33 - protein, 10 aa, Artificial Sequence
  Hu01 LFR4
FGGGTKVEIK

SEQ ID NO: 34 - protein, 107 aa, Artificial Sequence
  Mu01 VL
DIVMTQSHKFISTSVGDRVSITCKASQDVGTAVAWYQQIPGQSPKLLIYSASYRSTGIPDRFTGSGSGTDFSFIISSVQAEDLALYYCQHHYSAPWTFGGGTTLDIK

SEQ ID NO: 35 - protein, 107 aa, Artificial Sequence
  Hu01 VL
DIQMTQSPSSLSASVGDRVTITCKASQDVGTAVAWYQQKPGKAPKLLIYSASYRSTGVPSRFSGSGSGTDFTLTISSLQPEDFATYYCQHHYSAPWTFGGGTKVEIK

SEQ ID NO: 36 - protein, 107 aa, Artificial Sequence
  Mu01 VL; Hu01 VL
  misc_feature (3)..(3): Xaa = Gln or Val
  misc_feature (8)..(8): Xaa = His or Pro
  misc_feature (9)..(9): Xaa = Lys or Ser
  misc_feature (10)..(10): Xaa = Phe or Ser
  misc_feature (11)..(11): Xaa = Ile or Leu
  misc_feature (13)..(13): Xaa = Ala or Thr
  misc_feature (20)..(20): Xaa = Ser or Thr
  misc_feature (39)..(39): Xaa = Ile or Lys
  misc_feature (42)..(42): Xaa = Lys or Gln
  misc_feature (43)..(43): Xaa = Ala or Ser
  misc_feature (58)..(58): Xaa = Ile or Val
  misc_feature (60)..(60): Xaa = Asp or Ser
  misc_feature (63)..(63): Xaa = Ser or Thr
  misc_feature (72)..(72): Xaa = Ser or Thr
  misc_feature (73)..(73): Xaa = Phe or Leu
  misc_feature (74)..(74): Xaa = Ile or Thr
  misc_feature (78)..(78): Xaa = Leu or Val
  misc_feature (80)..(80): Xaa = Ala or Pro
  misc_feature (83)..(83): Xaa = Phe or Leu
  misc_feature (85)..(85): Xaa = Leu or Thr
  misc_feature (103)..(103): Xaa = Lys or Thr
  misc_feature (104)..(104): Xaa = Leu or Val
  misc_feature (105)..(105): Xaa = Asp or Glu
DIXMTQSXXXXSXSVGDRVXITCKASQDVGTAVAWYQQXPGXXPKLLIYSASYRSTGXPXRFXGSGSGTDFXXXISSXQXEDXAXYYCQHHYSAPWTFGGGTXXXIK

SEQ ID NO: 37 - protein, 15 aa, Artificial Sequence
  linker 1
GGGGSGGGGSGGGGS

SEQ ID NO: 38 - protein, 18 aa, Artificial Sequence
  linker 2
GSTSGSGKPGSGEGSTKG

SEQ ID NO: 39 - protein, 244 aa, Artificial Sequence
  Mu01 scFv VLVH
DIVMTQSHKFISTSVGDRVSITCKASQDVGTAVAWYQQIPGQSPKLLIYSASYRSTGIPDRFTGSGSGTDFSFIISSVQAEDLALYYCQHHYSAPWTFGGGTTLDIKGGGGSGGGGSGGGGSEVQLVESGGDLVRPGGSLQLSCAASGFTFSRNGMSWVRQTPDRRLEWVATVSSGGSYIYYADSVKGRFTISRDNARNTLYLQMSSLKSEDTAMYYCARQGTTALATRFFDVWGAGTTVTVSS

SEQ ID NO: 40 - protein, 244 aa, Artificial Sequence
  Hu01 scFv VLVH
DIQMTQSPSSLSASVGDRVTITCKASQDVGTAVAWYQQKPGKAPKLLIYSASYRSTGVPSRFSGSGSGTDFTLTISSLQPEDFATYYCQHHYSAPWTFGGGTKVEIKGGGGSGGGGSGGGGSEVQLVESGGGLVQPGGSLRLSCAASGFTFSRNGMSWVRQAPGKGLEWVATVSSGGSYIYYADSVKGRFTISRDNAKNSLYLQMNSLRAEDTAVYYCARQGTTALATRFFDVWGQGTLVTVSS

SEQ ID NO: 41 - protein, 244 aa, Artificial Sequence
  Mu01 scFv VLVH; Hu01 scFv VLVH
  misc_feature (3)..(3): Xaa = Gln or Val
  misc_feature (8)..(8): Xaa = His or Pro
  misc_feature (9)..(9): Xaa = Lys or Ser
  misc_feature (10)..(10): Xaa = Phe or Ser
  misc_feature (11)..(11): Xaa = Ile or Leu
  misc_feature (13)..(13): Xaa = Ala or Thr
  misc_feature (20)..(20): Xaa = Ser or Thr
  misc_feature (39)..(39): Xaa = Ile or Lys
  misc_feature (42)..(42): Xaa = Lys or Gln
  misc_feature (43)..(43): Xaa = Ala or Ser
  misc_feature (58)..(58): Xaa = Ile or Val
  misc_feature (60)..(60): Xaa = Asp or Ser
  misc_feature (63)..(63): Xaa = Ser or Thr
  misc_feature (72)..(72): Xaa = Ser or Thr
  misc_feature (73)..(73): Xaa = Phe or Leu
  misc_feature (74)..(74): Xaa = Ile or Thr
  misc_feature (78)..(78): Xaa = Leu or Val
  misc_feature (80)..(80): Xaa = Ala or Pro
  misc_feature (83)..(83): Xaa = Phe or Leu
  misc_feature (85)..(85): Xaa = Leu or Thr
  misc_feature (103)..(103): Xaa = Lys or Thr
  misc_feature (104)..(104): Xaa = Leu or Val
  misc_feature (105)..(105): Xaa = Asp or Glu
  misc_feature (132)..(132): Xaa = Asp or Gly
  misc_feature (135)..(135): Xaa = Gln or Arg
  misc_feature (141)..(141): Xaa = Gln or Arg
  misc_feature (162)..(162): Xaa = Ala or Thr
  misc_feature (164)..(164): Xaa = Asp or Gly
  misc_feature (165)..(165): Xaa = Lys or Arg
  misc_feature (166)..(166): Xaa = Gly or Arg
  misc_feature (198)..(198): Xaa = Lys or Arg
  misc_feature (200)..(200): Xaa = Ser or Thr
  misc_feature (206)..(206): Xaa = Asn or Ser
  misc_feature (209)..(209): Xaa = Lys or Arg
  misc_feature (210)..(210): Xaa = Ala or Ser
  misc_feature (215)..(215): Xaa = Met or Val
  misc_feature (236)..(236): Xaa = Ala or Gln
  misc_feature (239)..(239): Xaa = Leu or Thr
DIXMTQSXXXXSXSVGDRVXITCKASQDVGTAVAWYQQXPGXXPKLLIYSASYRSTGXPXRFXGSGSGTDFXXXISSXQXEDXAXYYCQHHYSAPWTFGGGTXXXIKGGGGSGGGGSGGGGSEVQLVESGGXLVXPGGSLXLSCAASGFTFSRNGMSWVRQXPXXXLEWVATVSSGGSYIYYADSVKGRFTISRDNAXNXLYLQMXSLXXEDTAXYYCARQGTTALATRFFDVWGXGTXVTVSS

SEQ ID NO: 42 - protein, 244 aa, Artificial Sequence
  Mu01 scFv VHVL
EVQLVESGGDLVRPGGSLQLSCAASGFTFSRNGMSWVRQTPDRRLEWVATVSSGGSYIYYADSVKGRFTISRDNARNTLYLQMSSLKSEDTAMYYCARQGTTALATRFFDVWGAGTTVTVSSGGGGSGGGGSGGGGSDIVMTQSHKFISTSVGDRVSITCKASQDVGTAVAWYQQIPGQSPKLLIYSASYRSTGIPDRFTGSGSGTDFSFIISSVQAEDLALYYCQHHYSAPWTFGGGTTLDIK

SEQ ID NO: 43 - protein, 244 aa, Artificial Sequence
  Hu01 scFv VHVL
EVQLVESGGGLVQPGGSLRLSCAASGFTFSRNGMSWVRQAPGKGLEWVATVSSGGSYIYYADSVKGRFTISRDNAKNSLYLQMNSLRAEDTAVYYCARQGTTALATRFFDVWGQGTLVTVSSGGGGSGGGGSGGGGSDIQMTQSPSSLSASVGDRVTITCKASQDVGTAVAWYQQKPGKAPKLLIYSASYRSTGVPSRFSGSGSGTDFTLTISSLQPEDFATYYCQHHYSAPWTFGGGTKVEIK

SEQ ID NO: 44 - protein, 244 aa, Artificial Sequence
  Mu01 scFv VHVL; Hu01 scFv VHVL
  misc_feature (10)..(10): Xaa = Asp or Gly
  misc_feature (13)..(13): Xaa = Gln or Arg
  misc_feature (19)..(19): Xaa = Gln or Arg
  misc_feature (40)..(40): Xaa = Ala or Thr
  misc_feature (42)..(42): Xaa = Asp or Gly
  misc_feature (43)..(43): Xaa = Lys or Arg
  misc_feature (44)..(44): Xaa = Gly or Arg
  misc_feature (76)..(76): Xaa = Lys or Arg
  misc_feature (78)..(78): Xaa = Ser or Thr
  misc_feature (84)..(84): Xaa = Asn or Ser
  misc_feature (87)..(87): Xaa = Lys or Arg
  misc_feature (88)..(88): Xaa = Ala or Ser
  misc_feature (93)..(93): Xaa = Met or Val
  misc_feature (114)..(114): Xaa = Ala or Gln
  misc_feature (117)..(117): Xaa = Leu or Thr
  misc_feature (140)..(140): Xaa = Gln or Val
  misc_feature (145)..(145): Xaa = His or Pro
  misc_feature (146)..(146): Xaa = Lys or Ser
  misc_feature (147)..(147): Xaa = Phe or Ser
  misc_feature (148)..(148): Xaa = Ile or Leu
  misc_feature (150)..(150): Xaa = Ala or Thr
  misc_feature (157)..(157): Xaa = Ser or Thr
  misc_feature (176)..(176): Xaa = Ile or Lys
  misc_feature (179)..(179): Xaa = Lys or Gln
  misc_feature (180)..(180): Xaa = Ala or Ser
  misc_feature (195)..(195): Xaa = Ile or Val
  misc_feature (197)..(197): Xaa = Asp or Ser
  misc_feature (200)..(200): Xaa = Ser or Thr
  misc_feature (209)..(209): Xaa = Ser or Thr
  misc_feature (210)..(210): Xaa = Phe or Leu
  misc_feature (211)..(211): Xaa = Ile or Thr
  misc_feature (215)..(215): Xaa = Leu or Val
  misc_feature (217)..(217): Xaa = Ala or Pro
  misc_feature (220)..(220): Xaa = Phe or Leu
  misc_feature (222)..(222): Xaa = Leu or Thr
  misc_feature (240)..(240): Xaa = Lys or Thr
  misc_feature (241)..(241): Xaa = Leu or Val
  misc_feature (242)..(242): Xaa = Asp or Glu
EVQLVESGGXLVXPGGSLXLSCAASGFTFSRNGMSWVRQXPXXXLEWVATVSSGGSYIYYADSVKGRFTISRDNAXNXLYLQMXSLXXEDTAXYYCARQGTTALATRFFDVWGXGTXVTVSSGGGGSGGGGSGGGGSDIXMTQSXXXXSXSVGDRVXITCKASQDVGTAVAWYQQXPGXXPKLLIYSASYRSTGXPXRFXGSGSGTDFXXXISSXQXEDXAXYYCQHHYSAPWTFGGGTXXXIK

SEQ ID NO: 45 - protein, 502 aa, Artificial Sequence
  Mu01 CAR VLVH;
MALPVTALLLPLALLLHAARPDIVMTQSHKFISTSVGDRVSITCKASQDVGTAVAWYQQIPGQSPKLLIYSASYRSTGIPDRFTGSGSGTDFSFIISSVQAEDLALYYCQHHYSAPWTFGGGTTLDIKGGGGSGGGGSGGGGSEVQLVESGGDLVRPGGSLQLSCAASGFTFSRNGMSWVRQTPDRRLEWVATVSSGGSYIYYADSVKGRFTISRDNARNTLYLQMSSLKSEDTAMYYCARQGTTALATRFFDVWGAGTTVTVSSFVPVFLPAKPTTTPAPRPPTPAPTIASQPLSLRPEACRPAAGGAVHTRGLDFACDIYIWAPLAGTCGVLLLSLVITLYCNHRNKRGRKKLLYIFKQPFMRPVQTTQEEDGCSCRFPEEEEGGCELRVKFSRSADAPAYQQGQNQLYNELNLGRREEYDVLDKRRGRDPEMGGKPRRKNPQEGLYNELQKDKMAEAYSEIGMKGERRRGKGHDGLYQGLSTATKDTYDALHMQALPPR

SEQ ID NO: 46 - protein, 502 aa, Artificial Sequence
  Hu01 CAR VHVL
MALPVTALLLPLALLLHAARPEVQLVESGGGLVQPGGSLRLSCAASGFTFSRNGMSWVRQAPGKGLEWVATVSSGGSYIYYADSVKGRFTISRDNAKNSLYLQMNSLRAEDTAVYYCARQGTTALATRFFDVWGQGTLVTVSSGGGGSGGGGSGGGGSDIQMTQSPSSLSASVGDRVTITCKASQDVGTAVAWYQQKPGKAPKLLIYSASYRSTGVPSRFSGSGSGTDFTLTISSLQPEDFATYYCQHHYSAPWTFGGGTKVEIKFVPVFLPAKPTTTPAPRPPTPAPTIASQPLSLRPEACRPAAGGAVHTRGLDFACDIYIWAPLAGTCGVLLLSLVITLYCNHRNKRGRKKLLYIFKQPFMRPVQTTQEEDGCSCRFPEEEEGGCELRVKFSRSADAPAYQQGQNQLYNELNLGRREEYDVLDKRRGRDPEMGGKPRRKNPQEGLYNELQKDKMAEAYSEIGMKGERRRGKGHDGLYQGLSTATKDTYDALHMQALPPR

SEQ ID NO: 47 - DNA, 366 bp, Artificial Sequence
  Mu01 VH nucleic acid sequence
gaggtgcagctggttgagtctggcggcgatcttgttagacctggcggaagcctgcagctgtcttgtgccgcttccggcttcaccttcagcagaaacggcatgagctgggtccgacagacccctgatagacggctggaatgggtcgccacagtgtctagcggcggcagctacatctactacgccgactctgtgaagggcagattcaccatctccagagacaacgcccggaacaccctgtacctgcagatgagcagcctgaagtccgaggacaccgccatgtactactgtgccagacagggcacaacagccctggccaccagattcttcgatgtgtggggagccggaaccaccgtgacagtctcttct

SEQ ID NO: 48 - DNA, 366 bp, Artificial Sequence
  Hu01 VH nucleic acid sequence
gaggtgcagctggtggagtctggcggcggactggtgcagcctggcggctctctgagactgtcttgtgccgcctccggcttcaccttcagtaggaatggcatgtcttgggtgaggcaggcccctggcaagggcctggagtgggtggccaccgttagtagtggtggtagttacatctactatgcagacagtgtgaaggggcggttcaccatctccagggacaacgccaagaactccctgtacctccagatgaactccctgagggccgaggataccgccgtgtactactgtgccagacaagggactacggcactagctacgaggttcttcgatgtctggggccagggcaccctggtgaccgtgtcctct

SEQ ID NO: 49 - DNA, 321 bp, Artificial Sequence
  Mu01 VL nucleic acid sequence
gacatcgtgatgacccagagccacaagttcatcagcaccagcgtgggcgacagagtgtccatcacctgtaaagccagccaggatgtgggaacagccgtggcctggtatcagcagatccctggccagtctcctaagctgctgatctacagcgccagctacagaagcacaggcatccccgatagattcaccggctctggcagcggcaccgacttcagctttatcatcagcagcgtgcaggccgaggatctggccctgtactattgccagcaccactactctgccccttggacctttggcggcggaaccacactggacatcaag

SEQ ID NO: 50 - DNA, 321 bp, Artificial Sequence
  Hu01 VL nucleic acid sequence
gacatccagatgacccagtccccctcttctctgtctgcctctgtgggcgacagagtgaccatcacctgtaaggccagtcaggatgtaggtactgctgtagcctggtatcagcagaagcctggcaaggctcccaagctgctgatctactcggcatcctaccggtccactggcgtgccttccagattctccggctctggctctggcaccgatttcaccctgaccatctcctccctccagcctgaggatttcgccacctactactgccagcaccattatagtgctccgtggacgtttggcggcggaacaaaggtggagatcaag

SEQ ID NO: 51 - DNA, 1506 bp, Artificial Sequence
  Mu01 CAR VLVH nucleic acid sequence;
atggccttaccagtgaccgccttgctcctgccgctggccttgctgctccacgccgccaggccggacatcgtgatgacccagagccacaagttcatcagcaccagcgtgggcgacagagtgtccatcacctgtaaagccagccaggatgtgggaacagccgtggcctggtatcagcagatccctggccagtctcctaagctgctgatctacagcgccagctacagaagcacaggcatccccgatagattcaccggctctggcagcggcaccgacttcagctttatcatcagcagcgtgcaggccgaggatctggccctgtactattgccagcaccactactctgccccttggacctttggcggcggaaccacactggacatcaagggaggcggaggttctggcggcggaggaagtggtggcggaggctctgaggtgcagctggttgagtctggcggcgatcttgttagacctggcggaagcctgcagctgtcttgtgccgcttccggcttcaccttcagcagaaacggcatgagctgggtccgacagacccctgatagacggctggaatgggtcgccacagtgtctagcggcggcagctacatctactacgccgactctgtgaagggcagattcaccatctccagagacaacgcccggaacaccctgtacctgcagatgagcagcctgaagtccgaggacaccgccatgtactactgtgccagacagggcacaacagccctggccaccagattcttcgatgtgtggggagccggaaccaccgtgacagtctcttctttcgtccccgtgttcctgcctgccaagccaacaactacccctgctccacgaccacctactccagcacctaccatcgcaagtcagcccctgtcactgcgacctgaggcttgccggccagcagctggaggagcagtgcacacccgaggcctggacttcgcatgcgatatctacatttgggcaccactggctggaacctgtggggtcctgctgctgagcctggtcatcaccctgtattgtaaccacagaaataaaagggggcgcaagaaactgctgtacatcttcaagcagccttttatgcgcccagtgcagacaactcaggaggaagacggatgctcttgtcggttcccagaggaggaggaaggaggctgcgagctgagagtgaagttcagccggagcgccgatgcaccagcatatcagcagggacagaatcagctgtacaacgagctgaatctgggcaggcgcgaggaatatgacgtgctggataagcgacgaggacgggaccccgaaatgggaggaaaacccagaaggaagaaccctcaggaggggctgtataatgaactgcagaaagacaagatggctgaggcatacagcgaaattggaatgaaaggagagcgccgacgggggaagggacacgatgggctgtaccagggactgtcaaccgccactaaagatacctacgacgcactgcacatgcaggctctgcccccaaga

SEQ ID NO: 52 - DNA, 1506 bp, Artificial Sequence
  Hu01 CAR VHVL nucleic acid sequence
atggccttaccagtgaccgccttgctcctgccgctggccttgctgctccacgccgccaggccggaggtgcagctggtggagtctggcggcggactggtgcagcctggcggctctctgagactgtcttgtgccgcctccggcttcaccttcagtaggaatggcatgtcttgggtgaggcaggcccctggcaagggcctggagtgggtggccaccgttagtagtggtggtagttacatctactatgcagacagtgtgaaggggcggttcaccatctccagggacaacgccaagaactccctgtacctccagatgaactccctgagggccgaggataccgccgtgtactactgtgccagacaagggactacggcactagctacgaggttcttcgatgtctggggccagggcaccctggtgaccgtgtcctctggaggcggaggttctggcggcggaggaagtggtggcggaggctctgacatccagatgacccagtccccctcttctctgtctgcctctgtgggcgacagagtgaccatcacctgtaaggccagtcaggatgtaggtactgctgtagcctggtatcagcagaagcctggcaaggctcccaagctgctgatctactcggcatcctaccggtccactggcgtgccttccagattctccggctctggctctggcaccgatttcaccctgaccatctcctccctccagcctgaggatttcgccacctactactgccagcaccattatagtgctccgtggacgtttggcggcggaacaaaggtggagatcaagttcgtccccgtgttcctgcctgccaagccaacaactacccctgctccacgaccacctactccagcacctaccatcgcaagtcagcccctgtcactgcgacctgaggcttgccggccagcagctggaggagcagtgcacacccgaggcctggacttcgcatgcgatatctacatttgggcaccactggctggaacctgtggggtcctgctgctgagcctggtcatcaccctgtattgtaaccacagaaataaaagggggcgcaagaaactgctgtacatcttcaagcagccttttatgcgcccagtgcagacaactcaggaggaagacggatgctcttgtcggttcccagaggaggaggaaggaggctgcgagctgagagtgaagttcagccggagcgccgatgcaccagcatatcagcagggacagaatcagctgtacaacgagctgaatctgggcaggcgcgaggaatatgacgtgctggataagcgacgaggacgggaccccgaaatgggaggaaaacccagaaggaagaaccctcaggaggggctgtataatgaactgcagaaagacaagatggctgaggcatacagcgaaattggaatgaaaggagagcgccgacgggggaagggacacgatgggctgtaccagggactgtcaaccgccactaaagatacctacgacgcactgcacatgcaggctctgcccccaaga

SEQ ID NO: 53 - protein, 6 aa, Artificial Sequence
  Hu07 HCDR1
TKYGVH

SEQ ID NO: 54 - protein, 16 aa, Artificial Sequence
  Hu07 HCDR2
GVKWAGGSTDYNSALM

SEQ ID NO: 55 - protein, 8 aa, Artificial Sequence
  Hu07 HCDR3
DHRDAMDY

SEQ ID NO: 56 - protein, 116 aa, Artificial Sequence
  Hu07 VH
EVQLVESGGGLVQPGGSLRLSCAASGFSLTKYGVHWVRQAPGKGLEWVGVKWAGGSTDYNSALMSRFTISKDNAKNSLYLQMNSLRAEDTAVYYCARDHRDAMDYWGQGTLVTVSS

SEQ ID NO: 57 - protein, 12 aa, Artificial Sequence
  Hu07 LCDR1
TASLSVSSTYLH

SEQ ID NO: 58 - protein, 7 aa, Artificial Sequence
  Hu07 LCDR2
STSNLAS

SEQ ID NO: 59 - protein, 9 aa, Artificial Sequence
  Hu07 LCDR3
HQYHRSPLT

SEQ ID NO: 60 - protein, 108 aa, Artificial Sequence
  Hu07 VL
DIQMTQSPSSLSASVGDRVTITCTASLSVSSTYLHWYQQKPGSSPKLWIYSTSNLASGVPSRFSGSGSGTSYTLTISSLQPEDFATYYCHQYHRSPLTFGGGTKVEIK

SEQ ID NO: 61 - protein, 239 aa, Artificial Sequence
  Hu07 scFv VHVL
EVQLVESGGGLVQPGGSLRLSCAASGFSLTKYGVHWVRQAPGKGLEWVGVKWAGGSTDYNSALMSRFTISKDNAKNSLYLQMNSLRAEDTAVYYCARDHRDAMDYWGQGTLVTVSSGGGGSGGGGSGGGGSDIQMTQSPSSLSASVGDRVTITCTASLSVSSTYLHWYQQKPGSSPKLWIYSTSNLASGVPSRFSGSGSGTSYTLTISSLQPEDFATYYCHQYHRSPLTFGGGTKVEIK

SEQ ID NO: 62 - protein, 239 aa, Artificial Sequence
  Hu07 scFv VLVH
DIQMTQSPSSLSASVGDRVTITCTASLSVSSTYLHWYQQKPGSSPKLWIYSTSNLASGVPSRFSGSGSGTSYTLTISSLQPEDFATYYCHQYHRSPLTFGGGTKVEIKGGGGSGGGGSGGGGSEVQLVESGGGLVQPGGSLRLSCAASGFSLTKYGVHWVRQAPGKGLEWVGVKWAGGSTDYNSALMSRFTISKDNAKNSLYLQMNSLRAEDTAVYYCARDHRDAMDYWGQGTLVTVSS

SEQ ID NO: 63 - DNA, 348 bp, Artificial Sequence
  Hu07 VH nucleotide sequence
gaagtacagctggttgagagtggcgggggtctcgtacagcccggcgggtctcttaggctctcctgtgctgcttctggtttctccttgactaaatacggggtacattgggttcgccaggcccctggcaaaggtcttgaatgggtgggcgtcaagtgggctggcggaagcactgattataattccgcattgatgtcccgattcactatttctaaggataatgccaagaacagtctctatttgcaaatgaactccctgagagcggaggatactgccgtttactactgtgcacgggatcaccgagacgctatggattactggggtcagggtaccctggtgaccgtaagctcc

SEQ ID NO: 64 - DNA, 324 bp, Artificial Sequence
  Hu07 VL nucleotide sequence
gacatacaaatgacacagtccccctcatccttgtctgcttccgtaggagaccgggttaccatcacgtgcaccgcttctttgtccgtttcaagtacctacctccactggtaccagcaaaaacccggcagcagccccaagttgtggatttactcaacttctaacttggcctcaggggtaccgtcaagatttagcggatctggcagtggcacgagttatactttgacgatatcaagccttcaaccggaggatttcgccacctattactgtcatcagtatcatcgaagccccttgacctttgggggagggacaaaagtggaaataaaa

SEQ ID NO: 65 - DNA, 648 bp, Artificial Sequence
  Hu07 scFv VHVL nucleotide sequence
gaagtacagctggttgagagtggcgggggtctcgtacagcccggcgggtctcttaggctctcctgtgctgcttctggtttctccttgactaaatacggggtacattgggttcgccaggcccctggcaaaggtcttgaatgggtgggcgtcaagtgggctggcggaagcactgattataattccgcattgatgtcccgattcactatttctaaggataatgccaagaacagtctctatttgcaaatgaactccctgagagcggaggatactgccgtttactactgtgcacgggatcaccgagacgctatggattactggggtcagggtaccctggtgaccgtaagctccgggggaggtggaagtggtggcggtggatctggtggcggcgggtcagacatacaaatgacacagtccccctcatccttgtctgcttccgtaggagaccgggttaccatcacgtgcaccgcttctttgtccgtttcaagtacctacctccactggtaccagcaaaaacccggcagcagccccaagttgtggatttactcaacttctaacttggcctcaggggtaccgtcaagatttagcggatctggcagtggcacgagttatactttgacgatatcaagccttcaaccggaggatttcgcc

SEQ ID NO: 66 - DNA, 717 bp, Artificial Sequence
  Hu07 scFv VLVH nucleotide sequence
gacatacaaatgacacagtccccctcatccttgtctgcttccgtaggagaccgggttaccatcacgtgcaccgcttctttgtccgtttcaagtacctacctccactggtaccagcaaaaacccggcagcagccccaagttgtggatttactcaacttctaacttggcctcaggggtaccgtcaagatttagcggatctggcagtggcacgagttatactttgacgatatcaagccttcaaccggaggatttcgccacctattactgtcatcagtatcatcgaagccccttgacctttgggggagggacaaaagtggaaataaaagggggaggtggaagtggtggcggtggatctggtggcggcgggtcagaagtacagctggttgagagtggcgggggtctcgtacagcccggcgggtctcttaggctctcctgtgctgcttctggtttctccttgactaaatacggggtacattgggttcgccaggcccctggcaaaggtcttgaatgggtgggcgtcaagtgggctggcggaagcactgattataattccgcattgatgtcccgattcactatttctaaggataatgccaagaacagtctctatttgcaaatgaactccctgagagcggaggatactgccgtttactactgtgcacgggatcaccgagacgctatggattactggggtcagggtaccctggtgaccgtaagctcc

SEQ ID NO: 67 - protein, 237 aa, Artificial Sequence
  CAR non-antigen binding domain amino acid sequence
FVPVFLPAKPTTTPAPRPPTPAPTIASQPLSLRPEACRPAAGGAVHTRGLDFACDIYIWAPLAGTCGVLLLSLVITLYCNHRNKRGRKKLLYIFKQPFMRPVQTTQEEDGCSCRFPEEEEGGCELRVKFSRSADAPAYQQGQNQLYNELNLGRREEYDVLDKRRGRDPEMGGKPRRKNPQEGLYNELQKDKMAEAYSEIGMKGERRRGKGHDGLYQGLSTATKDTYDALHMQALPPR

SEQ ID NO: 68 - DNA, 711 bp, Artificial Sequence
  CAR non-antigen binding domain DNA sequence
ttcgtccccgtgttcctgcctgccaagccaacaactacccctgctccacgaccacctactccagcacctaccatcgcaagtcagcccctgtcactgcgacctgaggcttgccggccagcagctggaggagcagtgcacacccgaggcctggacttcgcatgcgatatctacatttgggcaccactggctggaacctgtggggtcctgctgctgagcctggtcatcaccctgtattgtaaccacagaaataaaagggggcgcaagaaactgctgtacatcttcaagcagccttttatgcgcccagtgcagacaactcaggaggaagacggatgctcttgtcggttcccagaggaggaggaaggaggctgcgagctgagagtgaagttcagccggagcgccgatgcaccagcatatcagcagggacagaatcagctgtacaacgagctgaatctgggcaggcgcgaggaatatgacgtgctggataagcgacgaggacgggaccccgaaatgggaggaaaacccagaaggaagaaccctcaggaggggctgtataatgaactgcagaaagacaagatggctgaggcatacagcgaaattggaatgaaaggagagcgccgacgggggaagggacacgatgggctgtaccagggactgtcaaccgccactaaagatacctacgacgcactgcacatgcaggctctgcccccaaga

SEQ ID NO: 69 - protein, 21 aa, Artificial Sequence
  CD8A transmembrane domain
IYIWAPLAGTCGVLLLSLVIT

SEQ ID NO: 70 - protein, 21 aa, Artificial Sequence
  CD8B transmembrane domain
ITLGLLVAGVLVLLVSLGVAI

SEQ ID NO: 71 - protein, 27 aa, Artificial Sequence
  CD28 transmembrane domain
FWVLVVVGGVLACYSLLVTVAFIIFWV

SEQ ID NO: 72 - protein, 27 aa, Artificial Sequence
  4-1BB transmembrane domain
IISFFLALTSTALLFLLFFLTLRFSVV

SEQ ID NO: 73 - protein, 22 aa, Artificial Sequence
  CD4 transmembrane domain
MALIVLGGVAGLLLFIGLGIFF

SEQ ID NO: 74 - protein, 21 aa, Artificial Sequence
  CD27 transmembrane domain
ILVIFSGMFLVFTLAGALFLH

SEQ ID NO: 75 - protein, 21 aa, Artificial Sequence
  CD7 transmembrane domain
AALAVISFLLGLGLGVACVLA

SEQ ID NO: 76 - protein, 21 aa, Artificial Sequence
  PD-1 transmembrane domain
VGVVGGLLGSLVLLVWVLAVI

SEQ ID NO: 77 - protein, 23 aa, Artificial Sequence
  TRAC transmembrane domain
VIGFRILLLKVAGFNLLMTLRLW

SEQ ID NO: 78 - protein, 21 aa, Artificial Sequence
  TRBC transmembrane domain
ILLGKATLYAVLVSALVLMAM

SEQ ID NO: 79 - protein, 26 aa, Artificial Sequence
  CD3e transmembrane domain;CD3ε transmembrane domain
VMSVATIVIVDICITGGLLLLVYYWS

SEQ ID NO: 80 - protein, 21 aa, Artificial Sequence
  CD3ζ transmembrane domain
LCYLLDGILFIYGVILTALFL

SEQ ID NO: 81 - protein, 21 aa, Artificial Sequence
  CTLA-4 transmembrane domain
FLLWILAAVSSGLFFYSFLLT

SEQ ID NO: 82 - protein, 21 aa, Artificial Sequence
  LAG-3 transmembrane domain
LLFLILGVLSLLLLVTGAFGF

SEQ ID NO: 83 - protein, 30 aa, Artificial Sequence
  CD5 transmembrane domain
AGLAAGTVASIILALVLLVVLLVVCGPLAY

SEQ ID NO: 84 - protein, 21 aa, Artificial Sequence
  ICOS transmembrane domain
FWLPIGCAAFVVVCILGCILI

SEQ ID NO: 85 - protein, 21 aa, Artificial Sequence
  OX40 transmembrane domain
VAAILGLGLVLGLLGPLAILL

SEQ ID NO: 86 - protein, 21 aa, Artificial Sequence
  NKG2D transmembrane domain
PFFFCCFIAVAMGIRFIIMVA

SEQ ID NO: 87 - protein, 21 aa, Artificial Sequence
  2B4 transmembrane domain;CD244 transmembrane domain
FLVIIVILSALFLGTLACFCV

SEQ ID NO: 88 - protein, 21 aa, Artificial Sequence
  FcεRIγ transmembrane domain
LCYILDAILFLYGIVLTLLYC

SEQ ID NO: 89 - protein, 21 aa, Artificial Sequence
  BTLA transmembrane domain
LLPLGGLPLLITTCFCLFCCL

SEQ ID NO: 90 - protein, 21 aa, Artificial Sequence
  CD30 transmembrane domain
PVLFWVILVLVVVVGSSAFLL

SEQ ID NO: 91 - protein, 21 aa, Artificial Sequence
  GITR transmembrane domain
LGWLTVVLLAVAACVLLLTSA

SEQ ID NO: 92 - protein, 21 aa, Artificial Sequence
  HVEM transmembrane domain
WWFLSGSLVIVIVCSTVGLII

SEQ ID NO: 93 - protein, 21 aa, Artificial Sequence
  DAP10 transmembrane domain
LLAGLVAADAVASLLIVGAVF

SEQ ID NO: 94 - protein, 26 aa, Artificial Sequence
  CD2 transmembrane domain
IYLIIGICGGGSLLMVFVALLVFYIT

SEQ ID NO: 95 - protein, 23 aa, Artificial Sequence
  NKG2C transmembrane domain
LTAEVLGIICIVLMATVLKTIVL

SEQ ID NO: 96 - protein, 21 aa, Artificial Sequence
  LIGHT transmembrane domain
VGLGLLLLLMGAGLAVQGWFL

SEQ ID NO: 97 - protein, 21 aa, Artificial Sequence
  DAP12 transmembrane domain
GVLAGIVMGDLVLTVLIALAV

SEQ ID NO: 98 - protein, 24 aa, Artificial Sequence
  CD40L transmembrane domain;CD154 transmembrane domain
IFMYLLTVFLITQMIGSALFAVYL

SEQ ID NO: 99 - protein, 21 aa, Artificial Sequence
  TIM1 transmembrane domain
IYAGVCISVLVLLALLGVIIA

SEQ ID NO: 100 - protein, 21 aa, Artificial Sequence
  CD226 transmembrane domain
GGTVLLLLFVISITTIIVIFL

SEQ ID NO: 101 - protein, 21 aa, Artificial Sequence
  DR3 transmembrane domain
MFWVQVLLAGLVVPLLLGATL

SEQ ID NO: 102 - protein, 21 aa, Artificial Sequence
  CD45 transmembrane domain
ALIAFLAFLIIVTSIALLVVL

SEQ ID NO: 103 - protein, 21 aa, Artificial Sequence
  CD80 transmembrane domain
LLPSWAITLISVNGIFVICCL

SEQ ID NO: 104 - protein, 21 aa, Artificial Sequence
  CD86 transmembrane domain
WITAVLPTVIICVMVFCLILW

SEQ ID NO: 105 - protein, 21 aa, Artificial Sequence
  CD9 transmembrane domain1
LLFGFNFIFWLAGIAVLAIGL

SEQ ID NO: 106 - protein, 21 aa, Artificial Sequence
  CD9 transmembrane domain2
FYTGVYILIGAGALMMLVGFL

SEQ ID NO: 107 - protein, 24 aa, Artificial Sequence
  CD9 transmembrane domain3
MLGLFFGFLLVIFAIEIAAAIWGY

SEQ ID NO: 108 - protein, 26 aa, Artificial Sequence
  CD9 transmembrane domain4
IGAVGIGIAVVMIFGMIFSMILCCAI

SEQ ID NO: 109 - protein, 21 aa, Artificial Sequence
  CD16 transmembrane domain
VSFCLVMVLLFAVDTGLYFSV

SEQ ID NO: 110 - protein, 19 aa, Artificial Sequence
  CD22 transmembrane domain
VAVGLGSCLAILILAICGL

SEQ ID NO: 111 - protein, 23 aa, Artificial Sequence
  CD33 transmembrane domain
GAIGGAGVTALLALCLCLIFFIV

SEQ ID NO: 112 - protein, 21 aa, Artificial Sequence
  CD37 transmembrane domain1
FNLFFFVLGSLIFCFGIWILI

SEQ ID NO: 113 - protein, 15 aa, Artificial Sequence
  CD37 transmembrane domain2
VLAISGIFTMGIALL

SEQ ID NO: 114 - protein, 26 aa, Artificial Sequence
  CD37 transmembrane domain3
LLGLYFGMLLLLFATQITLGILISTQ

SEQ ID NO: 115 - protein, 25 aa, Artificial Sequence
  CD37 transmembrane domain4
LISIVGICLGVGLLELGFMTLSIFL

SEQ ID NO: 116 - protein, 21 aa, Artificial Sequence
  CD64 transmembrane domain
VLFYLAVGIMFLVNTVLWVTI

SEQ ID NO: 117 - protein, 21 aa, Artificial Sequence
  SLAM transmembrane domain
WAVYAGLLGGVIMILIMVVIL

SEQ ID NO: 118 - protein, 41 aa, Artificial Sequence
  CD28 intracellular co-stimulatory signaling domain
RSKRSRLLHSDYMNMTPRRPGPTRKHYQPYAPPRDFAAYRS

SEQ ID NO: 119 - protein, 42 aa, Artificial Sequence
  4-1BB intracellular co-stimulatory signaling domain
KRGRKKLLYIFKQPFMRPVQTTQEEDGCSCRFPEEEEGGCEL

SEQ ID NO: 120 - protein, 48 aa, Artificial Sequence
  CD27 intracellular co-stimulatory signaling domain
QRRKYRSNKGESPVEPAEPCHYSCPREEEGSTIPIQEDYRKPEPACSP

SEQ ID NO: 121 - protein, 116 aa, Artificial Sequence
  CD2 intracellular co-stimulatory signaling domain
KRKKQRSRRNDEELETRAHRVATEERGRKPHQIPASTPQNPATSQHPPPPPGHRSQAPSHRPPPPGHRVQHQPQKRPPAPSGTQVHQQKGPPLPRPRVQPKPPHGAAENSLSPSSN

SEQ ID NO: 122 - protein, 39 aa, Artificial Sequence
  CD7 intracellular co-stimulatory signaling domain
RTQIKKLCSWRDKNSAACVVYEDMSHSRCNTLSSPNQYQ

SEQ ID NO: 123 - protein, 32 aa, Artificial Sequence
  CD8A intracellular co-stimulatory signaling domain
LYCNHRNRRRVCKCPRPVVKSGDKPSLSARYV

SEQ ID NO: 124 - protein, 19 aa, Artificial Sequence
  CD8B intracellular co-stimulatory signaling domain
HLCCRRRRARLRFMKQFYK

SEQ ID NO: 125 - protein, 42 aa, Artificial Sequence
  OX40 intracellular co-stimulatory signaling domain
ALYLLRRDQRLPPDAHKPPGGGSFRTPIQEEQADAHSTLAKI

SEQ ID NO: 126 - protein, 61 aa, Artificial Sequence
  CD226 intracellular co-stimulatory signaling domain
NRRRRRERRDLFTESWDTQKAPNNYRSPISTSQPTNQSMDDTREDIYVNYPTFSRRPKTRV

SEQ ID NO: 127 - protein, 197 aa, Artificial Sequence
  DR3 intracellular co-stimulatory signaling domain
TYTYRHCWPHKPLVTADEAGMEALTPPPATHLSPLDSAHTLLAPPDSSEKICTVQLVGNSWTPGYPETQEALCPQVTWSWDQLPSRALGPAAAPTLSPESPAGSPAMMLQPGPQLYDVMDAVPARRWKEFVRTLGLREAEIEAVEVEIGRFRDQQYEMLKRWRQQQPAGLGAVYAALERMGLDGCVEDLRSRLQRGP

SEQ ID NO: 128 - protein, 77 aa, Artificial Sequence
  SLAM intracellular co-stimulatory signaling domain
QLRRRGKTNHYQTTVEKKSLTIYAQVQKPGPLQKKLDSFPAQDPCTTIYVAATEPVPESVQETNSITVYASVTLPES

SEQ ID NO: 129 - protein, 29 aa, Artificial Sequence
  ICAM-1 intracellular co-stimulatory signaling domain
NRQRKIKKYRLQQAQKGTPMKPNTQATPP

SEQ ID NO: 130 - protein, 51 aa, Artificial Sequence
  NKG2D intracellular co-stimulatory signaling domain
MGWIRGRRSRHSWEMSEFHNYNLDLKKSDFSTRWQKQRCPVVKSKCRENAS

SEQ ID NO: 131 - protein, 70 aa, Artificial Sequence
  NKG2C intracellular co-stimulatory signaling domain
MSKQRGTFSEVSLAQDPKRQQRKPKGNKSSISGTEQEIFQVELNLQNPSLNHQGIDKIYDCQGLLPPPEK

SEQ ID NO: 132 - protein, 47 aa, Artificial Sequence
  B7-H3 intracellular co-stimulatory signaling domain
CWRKIKQSCEEENAGAEDQDGEGEGSKTALQPLKHSDSKEDDGQEIA

SEQ ID NO: 133 - protein, 120 aa, Artificial Sequence
  2B4 intracellular co-stimulatory signaling domain;CD244 intracellular co-stimulatory signaling domain
WRRKRKEKQSETSPKEFLTIYEDVKDLKTRRNHEQEQTFPGGGSTIYSMIQSQSSAPTSQEPAYTLYSLIQPSRKSGSRKRNHSPSFNSTIYEVIGKSQPKAQNPARLSRKELENFDVYS

SEQ ID NO: 134 - protein, 42 aa, Artificial Sequence
  FcεRIγ intracellular co-stimulatory signaling domain;FcεRIγ intracellular signaling domain
RLKIQVRKAAITSYEKSDGVYTGLSTRNQETYETLKHEKPPQ

SEQ ID NO: 135 - protein, 111 aa, Artificial Sequence
  BTLA intracellular co-stimulatory signaling domain
RRHQGKQNELSDTAGREINLVDAHLKSEQTEASTRQNSQVLLSETGIYDNDPDLCFRMQEGSEVYSNPCLEENKPGIVYASLNHSVIGPNSRLARNVKEAPTEYASICVRS

SEQ ID NO: 136 - protein, 58 aa, Artificial Sequence
  GITR intracellular co-stimulatory signaling domain
QLGLHIWQLRSQCMWPRETQLLLEVPPSTEDARSCQFPEEERGERSAEEKGRLGDLWV

SEQ ID NO: 137 - protein, 60 aa, Artificial Sequence
  HVEM intracellular co-stimulatory signaling domain
CVKRRKPRGDVVKVIVSVQRKRQEAEGEATVIEALQAPPDVTTVAVEETIPSFTGRSPNH

SEQ ID NO: 138 - protein, 24 aa, Artificial Sequence
  DAP10 intracellular co-stimulatory signaling domain;DAP10 intracellular signaling domain
LCARPRRSPAQEDGKVYINMPGRG

SEQ ID NO: 139 - protein, 52 aa, Artificial Sequence
  DAP12 intracellular co-stimulatory signaling domain;DAP-12 intracellular signaling domain
YFLGRLVPRGRGAAEAATRKQRITETESPYQELQGQRSDVYSDLNTQRPYYK

SEQ ID NO: 140 - protein, 189 aa, Artificial Sequence
  CD30 intracellular co-stimulatory signaling domain
CHRRACRKRIRQKLHLCYPVQTSQPKLELVDSRPRRSSTQLRSGASVTEPVAEERGLMSQPLMETCHSVGAAYLESLPLQDASPAGGPSSPRDLPEPRVSTEHTNNKIEKIYIMKADTVIVGTVKAELPEGRGLAGPAEPELEEELEADHTPHYPEQETEPPLGSCSDVMLSVEEEGKEDPLPTAASGK

SEQ ID NO: 141 - protein, 62 aa, Artificial Sequence
  CD40 intracellular co-stimulatory signaling domain
KKVAKKPTNKAPHPKQEPQEINFPDDLPGSNTAAPVQETLHGCQPVTQEDGKESRISVQERQ

SEQ ID NO: 142 - protein, 22 aa, Artificial Sequence
  CD40L intracellular co-stimulatory signaling domain
MIETYNQTSPRSAATGLPISMK

SEQ ID NO: 143 - protein, 48 aa, Artificial Sequence
  TIM1 intracellular co-stimulatory signaling domain
KKYFFKKEVQQLSVSFSSLQIKALQNAVEKEVQAEDNIYIENSLYATD

SEQ ID NO: 144 - protein, 97 aa, Artificial Sequence
  PD-1 intracellular co-stimulatory signaling domain
CSRAARGTIGARRTGQPLKEDPSAVPVFSVDYGELDFQWREKTPEPPVPCVPEQTEYATIVFPSGMGTSSPARRGSADGPRSAQPLRPEDGHCSWPL

SEQ ID NO: 145 - protein, 59 aa, Artificial Sequence
  LFA-1 intracellular co-stimulatory signaling domain
YKVGFFKRNLKEKMEAGRGVPNGIPAEDSEQLASGQEAGDPGCLKPLHEKDSESGGGKD

SEQ ID NO: 146 - protein, 182 aa, Artificial Sequence
  LIGHT intracellular co-stimulatory signaling domain
LQLHWRLGEMVTRLPDGPAGSWEQLIQERRSHEVNPAAHLTGANSSLTGSGGPLLWETQLGLAFLRGLSYHDGALVVTKAGYYYIYSKVQLGGVGCPLGLASTITHGLYKRTPRYPEELELLVSQQSPCGRATSSSRVWWDSSFLGGVVHLEAGEKVVVRVLDERLVRLRDGTRSYFGAFMV

SEQ ID NO: 147 - protein, 98 aa, Artificial Sequence
  JAML intracellular co-stimulatory signaling domain
KKTCGNKSSVNSTVLVKNTKKTNPEIKEKPCHFERCEGEKHIYSPIIVREVIEEEEPSEKSEATYMTMHPVWPSLRSDRNNSLEKKSGGGMPKTQQAF

SEQ ID NO: 148 - protein, 107 aa, Artificial Sequence
  CD100 intracellular co-stimulatory signaling domain
YKGYLPRQCLKFRSALLIGKKKPKSDFCDREQSLKETLVEPGSFSQQNGEHPKPALDTGYETEQDTITSKVPTDREDSQRIDDLSARDKPFDVKCELKFADSDADGD

SEQ ID NO: 149 - protein, 38 aa, Artificial Sequence
  ICOS intracellular co-stimulatory signaling domain
CWLTKKKYSSSVHDPNGEYMFMRAVNTAKKSRLTDVTL

SEQ ID NO: 150 - protein, 296 aa, Artificial Sequence
  MyD88 intracellular co-stimulatory signaling domain
MAAGGPGAGSAAPVSSTSSLPLAALNMRVRRRLSLFLNVRTQVAADWTALAEEMDFEYLEIRQLETQADPTGRLLDAWQGRPGASVGRLLELLTKLGRDDVLLELGPSIEEDCQKYILKQQQEEAEKPLQVAAVDSSVPRTAELAGITTLDDPLGHMPERFDAFICYCPSDIQFVQEMIRQLEQTNYRLKLCVSDRDVLPGTCVWSIASELIEKRCRRMVVVVSDDYLQSKECDFQTKFALSLSPGAHQKRLIPIKYKAMKKEFPSILRFITVCDYTNPCTKSWFWTRLAKALSLP

SEQ ID NO: 151 - protein, 113 aa, Artificial Sequence
  CD3ζ intracellular signaling domain
RVKFSRSADAPAYQQGQNQLYNELNLGRREEYDVLDKRRGRDPEMGGKPQRRKNPQEGLYNELQKDKMAEAYSEIGMKGERRRGKGHDGLYQGLSTATKDTYDALHMQALPPR

SEQ ID NO: 152 - protein, 45 aa, Artificial Sequence
  CD3δ intracellular signaling domain
GHETGRLSGAADTQALLRNDQVYQPLRDRDDAQYSHLGGNWARNK

SEQ ID NO: 153 - protein, 45 aa, Artificial Sequence
  CD3γ intracellular signaling domain
GQDGVRQSRASDKQTLLPNDQLYQPLKDREDDQYSHLQGNQLRRN

SEQ ID NO: 154 - protein, 55 aa, Artificial Sequence
  CD3ε intracellular signaling domain
KNRKAKAKPVTRGAGAGGRQRGQNKERPPPVPNPDYEPIRKGQRDLYSGLNQRRI

SEQ ID NO: 155 - protein, 61 aa, Artificial Sequence
  CD79a intracellular signaling domain
RKRWQNEKLGLDAGDEYEDENLYEGLNLDDCSMYEDISRGLQGTYQDVGSLNIGDVQLEKP

SEQ ID NO: 156 - protein, 49 aa, Artificial Sequence
  CD79b intracellular signaling domain
LDKDDSKAGMEEDHTYEGLDIDQTATYEDIVTLRTGEVKWSVGEHPGQE

SEQ ID NO: 157 - protein, 44 aa, Artificial Sequence
  FceRIβ intracellular signaling domain
ICGAGEELKGNKVPEDRVYEELNIYSATYSELEDPGEMSPPIDL

SEQ ID NO: 158 - protein, 77 aa, Artificial Sequence
  FcγRIIa intracellular signaling domain
CRKKRISANSTDPVKAAQFEPPGRQMIAIRKRQLEETNNDYETADGGYMTLNPRAPTDDDKNIYLTLPPNDHVNSNN

SEQ ID NO: 159 - protein, 58 aa, Artificial Sequence
  bovine leukemia virus gp30 intracellular signaling domain
KCLTSRLLKLLRQAPHFPEISFPPKPDSDYQALLPSAPEIYSHLSPTKPDYINLRPCP

SEQ ID NO: 160 - protein, 123 aa, Artificial Sequence
  Epstein-Barr Virus (EBV) LMP2A intracellular signaling domain
MGSLEMVPMGAGPPSPGGDPDGYDGGNNSQYPSASGSSGNTPTPPNDEERESNEEPPPPYEDPYWGNGDRHSDYQPLGTQDQSLYLGLQHDGNDGLPPPPYSPRDDSSQHIYEEAGRGSMNPV

SEQ ID NO: 161 - protein, 260 aa, Artificial Sequence
  simian immunodeficiency virus PBj14 Nef intracellular signaling domain
GGVTSKKQRRRGGNLYERLLQARGETYGRLWEGLEGEYSQSQDASGKGLSSLSCEPQKYCEGQFMNTPWRNPATERAKLDYRQQNMDDVDSADLVGCPVSPRVPVRIMTYKLAIDMSHFIKEKGGLEGIYYSDRRHKILDLYLEKEEGIIPDWQNYTAGPGIRYPMFFGWLWKLVPVNVSDEAQEDETHYLMHPAQTSQWDDPWGEVLAWKFDPKLAYNYKAFVEHPEEFGSQSGLSKEEVQRRLTARGLLKMADKKKTS

SEQ ID NO: 162 - protein, 134 aa, Artificial Sequence
  CD28  hinge region
NKILVKQSPMLVAYDNAVNLSCKYSYNLFSREFRASLHKGLDSAVEVCVVYGNYSQQLQVYSKTGFNCDGKLGNESVTFYLQNLYVNQTDIYFCKIEVMYPPPYLDNEKSNGTIIHVKGKHLCPSPLFPGPSKP

SEQ ID NO: 163 - protein, 220 aa, Artificial Sequence
  IgG1 hinge region
PCPAPELLGGPSVFLFPPKPKDTLMISRTPEVTCVVVDVSHEDPEVKFNWYVDGVEVHNAKTKPREEQYNSTYRVVSVLTVLHQDWLNGKEYKCKVSNKALPAPIEKTISKAKGQPREPQVYTLPPSRDELTKNQVSLTCLVKGFYPSDIAVEWESNGQPENNYKTTPPVLDSDGSFFLYSKLTVDKSRWQQGNVFSCSVMHEALHNHYTQKSLSLSPGK

SEQ ID NO: 164 - protein, 217 aa, Artificial Sequence
  IgG4 hinge region
APEFLGGPSVFLFPPKPKDTLMISRTPEVTCVVVDVSQEDPEVQFNWYVDGVEVHNAKTKPREEQFNSTYRVVSVLTVLHQDWLNGKEYKCKVSNKGLPSSIEKTISKAKGQPREPQVYTLPPSQEEMTKNQVSLTCLVKGFYPSDIAVEWESNGQPENNYKTTPPVLDSDGSFFLYSRLTVDKSRWQEGNVFSCSVMHEALHNHYTQKSLSLSLGK

SEQ ID NO: 165 - protein, 223 aa, Artificial Sequence
  IgD hinge region
CPSHTQPLGVYLLTPAVQDLWLRDKATFTCFVVGSDLKDAHLTWEVAGKVPTGGVEEGLLERHSNGSQSQHSRLTLPRSLWNAGTSVTCTLNHPSLPPQRLMALREPAQAPVKLSLNLLASSDPPEAASWLLCEVSGFSPPNILLMWLEDQREVNTSGFAPARPPPQPRSTTFWAWSVLRVPAPPSPQPATYTCVVSHEDSRTLLNASRSLEVSYVTDHGPMK

SEQ ID NO: 166 - protein, 163 aa, Artificial Sequence
  4-1BB hinge region
LQDPCSNCPAGTFCDNNRNQICSPCPPNSFSSAGGQRTCDICRQCKGVFRTRKECSSTSNAECDCTPGFHCLGAGCSMCEQDCKQGQELTKKGCKDCCFGTFNDQKRGICRPWTNCSLDGKSVLVNGTKERDVVCGPSPADLSPGASSVTPPAPAREPGHSPQ

SEQ ID NO: 167 - protein, 371 aa, Artificial Sequence
  CD4 hinge region
KKVVLGKKGDTVELTCTASQKKSIQFHWKNSNQIKILGNQGSFLTKGPSKLNDRADSRRSLWDQGNFPLIIKNLKIEDSDTYICEVEDQKEEVQLLVFGLTANSDTHLLQGQSLTLTLESPPGSSPSVQCRSPRGKNIQGGKTLSVSQLELQDSGTWTCTVLQNQKKVEFKIDIVVLAFQKASSIVYKKEGEQVEFSFPLAFTVEKLTGSGELWWQAERASSSKSWITFDLKNKEVSVKRVTQDPKLQMGKKLPLHLTLPQALPQYAGSGNLTLALEAKTGKLHQEVNLVVMRATQLQKNLTCEVWGPTSPKLMLSLKLENKEAKVSKREKAVWVLNPEAGMWQCLLSDSGQVLLESNIKVLPTWSTPVQP

SEQ ID NO: 168 - protein, 172 aa, Artificial Sequence
  CD27 hinge region
ATPAPKSCPERHYWAQGKLCCQMCEPGTFLVKDCDQHRKAAQCDPCIPGVSFSPDHHTRPHCESCRHCNSGLLVRNCTITANAECACRNGWQCRDKECTECDPLPNPSLTARSSQALSPHPQPTHLPYVSEMLEARTAGHMQTLADFRQLPARTLSTHWPPQRSLCSSDFIR

SEQ ID NO: 169 - protein, 155 aa, Artificial Sequence
  CD7 hinge region
AQEVQQSPHCTTVPVGASVNITCSTSGGLRGIYLRQLGPQPQDIIYYEDGVVPTTDRRFRGRIDFSGSQDNLTITMHRLQLSDTGTYTCQAITEVNVYGSGTLVLVTEEQSQGWHRCSDAPPRASALPAPPTGSALPDPQTASALPDPPAASALP

SEQ ID NO: 170 - protein, 161 aa, Artificial Sequence
  CD8A hinge region
SQFRVSPLDRTWNLGETVELKCQVLLSNPTSGCSWLFQPRGAAASPTFLLYLSQNKPKAAEGLDTQRFSGKRLGDTFVLTLSDFRRENEGYYFCSALSNSIMYFSHFVPVFLPAKPTTTPAPRPPTPAPTIASQPLSLRPEACRPAAGGAVHTRGLDFACD

SEQ ID NO: 171 - protein, 147 aa, Artificial Sequence
  PD-1 hinge region
FLDSPDRPWNPPTFSPALLVVTEGDNATFTCSFSNTSESFVLNWYRMSPSNQTDKLAAFPEDRSQPGQDCRFRVTQLPNGRDFHMSVVRARRNDSGTYLCGAISLAPKAQIKESLRAELRVTERRAEVPTAHPSPSPRPAGQFQTLV

SEQ ID NO: 172 - protein, 120 aa, Artificial Sequence
  ICOS hinge region
EINGSANYEMFIFHNGGVQILCKYPDIVQQFKMQLLKGGQILCDLTKTKGSGNTVSIKSLKFCHSQLSNNSVSFFLYNLDHSHANYYFCNLSIFDPPPFKVTLTGGYLHIYESQLCCQLK

SEQ ID NO: 173 - protein, 133 aa, Artificial Sequence
  OX40 hinge region
QVSHRYPRIQSIKVQFTEYKKEKGFILTSQKEDEIMKVQNNSVIINCDGFYLISLKGYFSQEVNISLHYQKDEEPLFQLKKVRSVNSLMVASLTYKDKVYLNVTTDNTSLDDFHVNGGELILIHQNPGEFCVL

SEQ ID NO: 174 - protein, 144 aa, Artificial Sequence
  NKG2D hinge region
IWSAVFLNSLFNQEVQIPLTESYCGPCPKNWICYKNNCYQFFDESKNWYESQASCMSQNASLLKVYSKEDQDLLKLVKSYHWMGLVHIPTNGSWQWEDGSILSPNLLTIIEMQKGDCALYASSFKGYIENCSTPNTYICMQRTV

SEQ ID NO: 175 - protein, 138 aa, Artificial Sequence
  NKG2C hinge region
IPFLEQNNSSPNTRTQKARHCGHCPEEWITYSNSCYYIGKERRTWEESLLACTSKNSSLLSIDNEEEMKFLASILPSSWIGVFRNSSHHPWVTINGLAFKHKIKDSDNAELNCAVLQVNRLKSAQCGSSMIYHCKHKL

SEQ ID NO: 176 - protein, 5 aa, Artificial Sequence
  FcεRIγ hinge region
LGEPQ

SEQ ID NO: 177 - protein, 127 aa, Artificial Sequence
  BTLA hinge region
KESCDVQLYIKRQSEHSILAGDPFELECPVKYCANRPHVTWCKLNGTTCVKLEDRQTSWKEEKNISFFILHFEPVLPNDNGSYRCSANFQSNLIESHSTTLYVTDVKSASERPSKDEMASRPWLLYR

SEQ ID NO: 178 - protein, 137 aa, Artificial Sequence
  GITR hinge region
QRPTGGPGCGPGRLLLGTGTDARCCRVHTTRCCRDYPGEECCSEWDCMCVQPEFHCGDPCCTTCRHHPCPPGQGVQSQGKFSFGFQCIDCASGTFSGGHEGHCKPWTDCTQFGFLTVFPGNKTHNAVCVPGSPPAEP

SEQ ID NO: 179 - protein, 30 aa, Artificial Sequence
  DAP10 hinge region
QTTPGERSSLPAFYPGTSGSCSGCGSLSLP

SEQ ID NO: 180 - protein, 275 aa, Artificial Sequence
  TIM1 hinge region
SVKVGGEAGPSVTLPCHYSGAVTSMCWNRGSCSLFTCQNGIVWTNGTHVTYRKDTRYKLLGDLSRRDVSLTIENTAVSDSGVYCCRVEHRGWFNDMKITVSLEIVPPKVTTTPIVTTVPTVTTVRTSTTVPTTTTVPMTTVPTTTVPTTMSIPTTTTVLTTMTVSTTTSVPTTTSIPTTTSVPVTTTVSTFVPPMPLPRQNHEPVATSPSSPQPAETHPTTLQGAIRREPTSSPLYSYTTDGNDTVTESSDGLWNNNQTQLFLEHSLLTANTTKG

SEQ ID NO: 181 - protein, 217 aa, Artificial Sequence
  SLAM hinge region
ASYGTGGRMMNCPKILRQLGSKVLLPLTYERINKSMNKSIHIVVTMAKSLENSVENKIVSLDPSEAGPPRYLGDRYKFYLENLTLGIRESRKEDEGWYLMTLEKNVSVQRFCLQLRLYEQVSTPEIKVLNKTQENGTCTLILGCTVEKGDHVAYSWSEKAGTHPLNPANSSHLLSLTLGPQHADNIYICTVSNPISNNSQTFSPWPGCRTDPSETKP

SEQ ID NO: 182 - protein, 367 aa, Artificial Sequence
  CD30 hinge region
FPQDRPFEDTCHGNPSHYYDKAVRRCCYRCPMGLFPTQQCPQRPTDCRKQCEPDYYLDEADRCTACVTCSRDDLVEKTPCAWNSSRVCECRPGMFCSTSAVNSCARCFFHSVCPAGMIVKFPGTAQKNTVCEPASPGVSPACASPENCKEPSSGTIPQAKPTPVSPATSSASTMPVRGGTRLAQEAASKLTRAPDSPSSVGRPSSDPGLSPTQPCPEGSGDCRKQCEPDYYLDEAGRCTACVSCSRDDLVEKTPCAWNSSRTCECRPGMICATSATNSCARCVPYPICAAETVTKPQDMAEKDTTFEAPPLGTQPDCNPTPENGEAPASTSPTQSLLVDSQASKTLPIPTSAPVALSSTGKPVLDAG

SEQ ID NO: 183 - protein, 37 aa, Artificial Sequence
  LIGHT hinge region
MEESVVRPSVFVVDGQTDIPFTRLGRSHRRQSCSVAR

SEQ ID NO: 184 - protein, 21 aa, Artificial Sequence
  CD8A signal peptide amino acid sequence
MALPVTALLLPLALLLHAARP

SEQ ID NO: 185 - DNA, 63 bp, Artificial Sequence
  CD8A signal peptide nucleic acid sequence
atggccttaccagtgaccgccttgctcctgccgctggccttgctgctccacgccgccaggccg

SEQ ID NO: 186 - RNA, 20 nt, Artificial Sequence
  TRAC sg9
agagucucucagcugguaca

SEQ ID NO: 187 - RNA, 20 nt, Artificial Sequence
  TRAC sg10
ugugcuagacaugaggucua

SEQ ID NO: 188 - RNA, 20 nt, Artificial Sequence
  TRAC sg11
cucucagcugguacacggca

SEQ ID NO: 189 - RNA, 20 nt, Artificial Sequence
  TRAC sg12
acacggcagggucaggguuc

SEQ ID NO: 190 - RNA, 20 nt, Artificial Sequence
  TRAC sg13
agcugguacacggcaggguc

SEQ ID NO: 191 - RNA, 20 nt, Artificial Sequence
  TRAC sg14
gagaaucaaaaucggugaau

SEQ ID NO: 192 - RNA, 20 nt, Artificial Sequence
  TRAC sg15
gacaccuucuuccccagccc

SEQ ID NO: 193 - RNA, 20 nt, Artificial Sequence
  TRAC sg16
ucucucagcugguacacggc

SEQ ID NO: 194 - RNA, 20 nt, Artificial Sequence
  TRAC sg17
gcugguacacggcaggguca

SEQ ID NO: 195 - RNA, 20 nt, Artificial Sequence
  TRAC sg18
aaagucagauuuguugcucc

SEQ ID NO: 196 - RNA, 20 nt, Artificial Sequence
  TRAC sg19
cuggggaagaaggugucuuc

SEQ ID NO: 197 - RNA, 20 nt, Artificial Sequence
  TRAC sg20
uggauuuagagucucucagc

SEQ ID NO: 198 - RNA, 20 nt, Artificial Sequence
  TRAC sg21
agagcaacagugcuguggcc

SEQ ID NO: 199 - RNA, 20 nt, Artificial Sequence
  TRAC sg22
cuucaagagcaacagugcug

SEQ ID NO: 200 - RNA, 20 nt, Artificial Sequence
  TRAC sg23
auuuguuugagaaucaaaau

SEQ ID NO: 201 - RNA, 20 nt, Artificial Sequence
  HLA-A02 sg10
cccucguccugcuacucucg

SEQ ID NO: 202 - RNA, 20 nt, Artificial Sequence
  HLA-A02 sg2
cguacuggugguacccgcgg

SEQ ID NO: 203 - RNA, 20 nt, Artificial Sequence
  HLA-A02 sg5
cugaccaugaagccacccug

SEQ ID NO: 204 - RNA, 20 nt, Artificial Sequence
  HLA-A02 sg14
agacucaccgaguggaccug

SEQ ID NO: 205 - RNA, 20 nt, Artificial Sequence
  HLA-A02 sg21
ggacccuccugcucuaucca

SEQ ID NO: 206 - RNA, 20 nt, Artificial Sequence
  HLA-A02 sg23
gauguaauccuugccgucgu

SEQ ID NO: 207 - RNA, 20 nt, Artificial Sequence
  HLA-A02 sg26
ccugcgcucuuggaccgcgg

SEQ ID NO: 208 - RNA, 20 nt, Artificial Sequence
  HLA-A02 sg29
ccucguccugcuacucucgg

SEQ ID NO: 209 - RNA, 20 nt, Artificial Sequence
  HLA-A02 sg30
aacccucguccugcuacucu

SEQ ID NO: 210 - RNA, 20 nt, Artificial Sequence
  HLA-A02 sg31
gaggguucggggcgccauga

SEQ ID NO: 211 - RNA, 20 nt, Artificial Sequence
  HLA-A02 sg32
ccugcuacucucgggggcuc

SEQ ID NO: 212 - RNA, 20 nt, Artificial Sequence
  HLA-A02 sg33
cugguuguaguagccgcgca

SEQ ID NO: 213 - RNA, 20 nt, Artificial Sequence
  HLA-A02 sg34
uagcccacugcgaugaagcg

SEQ ID NO: 214 - RNA, 20 nt, Artificial Sequence
  HLA-A02 sg35
guggaccuggggacccugcg

SEQ ID NO: 215 - RNA, 20 nt, Artificial Sequence
  HLA-A02 sg36
uggacgacacgcaguucgug

SEQ ID NO: 216 - RNA, 20 nt, Artificial Sequence
  HLA-A02 sg37
acagacucaccgaguggacc

SEQ ID NO: 217 - RNA, 20 nt, Artificial Sequence
  HLA-A02 sg38
gcaggaggguccggaguauu

SEQ ID NO: 218 - RNA, 20 nt, Artificial Sequence
  HLA-A02 sg39
aguauugggacggggagaca

SEQ ID NO: 219 - RNA, 20 nt, Artificial Sequence
  HLA-A02 sg40
cucagaccaccaagcacaag

SEQ ID NO: 220 - RNA, 20 nt, Artificial Sequence
  HLA-A02 sg41
ccgccgcgguccaagagcgc

SEQ ID NO: 221 - RNA, 20 nt, Artificial Sequence
  HLA-A02 sg42
cucuuggaccgcggcggaca

SEQ ID NO: 222 - RNA, 20 nt, Artificial Sequence
  HLA-A02 sg43
ggauuacaucgcccugaaag

SEQ ID NO: 223 - RNA, 20 nt, Artificial Sequence
  HLA-A11 sg8-3
cccccgagaguagcaggagg

SEQ ID NO: 224 - RNA, 20 nt, Artificial Sequence
  HLA-A11 sg9-3
aguagcaggaggaggguucg

SEQ ID NO: 225 - RNA, 20 nt, Artificial Sequence
  HLA-A11 sg10-3
cccuccuccugcuacucucg

SEQ ID NO: 226 - RNA, 20 nt, Artificial Sequence
  HLA-A11 sg11-3
ccccgagaguagcaggagga

SEQ ID NO: 227 - RNA, 20 nt, Artificial Sequence
  HLA-A11 sg14-3
agacugaccgaguggaccug

SEQ ID NO: 228 - RNA, 20 nt, Artificial Sequence
  HLA-A11 sg16-3
ggggccggaguauugggacc

SEQ ID NO: 229 - RNA, 20 nt, Artificial Sequence
  HLA-A11 sg20-3
ccacucggucagucugugac

SEQ ID NO: 230 - RNA, 20 nt, Artificial Sequence
  HLA-A11 sg21-3
uggauagagcaggaggggcc

SEQ ID NO: 231 - RNA, 20 nt, Artificial Sequence
  HLA-A11 sg28-3
ugccgucguaggcguccugc

SEQ ID NO: 232 - RNA, 20 nt, Artificial Sequence
  HLA-A11 Rsg2
cguccugccgguacccgcgg

SEQ ID NO: 233 - RNA, 20 nt, Artificial Sequence
  HLA-A11 sg21
ggccccuccugcucuaucca

SEQ ID NO: 234 - RNA, 20 nt, Artificial Sequence
  HLA-A24 sg12-2
ccuggcccugacccagaccu

SEQ ID NO: 235 - RNA, 20 nt, Artificial Sequence
  HLA-A24 sg13-2
cccuggcccugacccagacc

SEQ ID NO: 236 - RNA, 20 nt, Artificial Sequence
  HLA-A24 sg14-2
agacugaccgagagaaccug

SEQ ID NO: 237 - RNA, 20 nt, Artificial Sequence
  HLA-A24 sg16-2
ggggccggaguauugggacg

SEQ ID NO: 238 - RNA, 20 nt, Artificial Sequence
  HLA-A24 sg20-2
ucucucggucagucugugag

SEQ ID NO: 239 - RNA, 20 nt, Artificial Sequence
  HLA-A24 sg21-2
ggccccuccugcucuaucca

SEQ ID NO: 240 - RNA, 20 nt, Artificial Sequence
  HLA-A24 sg22-2
aggcguacuggugguacccg

SEQ ID NO: 241 - RNA, 20 nt, Artificial Sequence
  HLA-A24 sg25-2
cugagccgccauguccgccg

SEQ ID NO: 242 - RNA, 21 nt, Artificial Sequence
  HLA-A-homo-551
gcggagcaguugagagccuac

SEQ ID NO: 243 - RNA, 21 nt, Artificial Sequence
  HLA-A-homo-NEG
gcucagaucaccaagcgcaag

SEQ ID NO: 244 - RNA, 21 nt, Artificial Sequence
  TRAC-homo-375
gaaaguggccggguuuaaucu

SEQ ID NO: 245 - RNA, 21 nt, Artificial Sequence
  TRAC-homo-NEG
gaaacagauacgaaccuaaac